European Patent Specification EP 3 419 993 B1, published September 6, 2023. Title: Enhancing Photosynthesis. Applicant: University of Essex Enterprises Limited. The sequence listing filed with the application follows.

SEQUENCE LISTING (5 sequences)

SEQ ID NO: 1 - protein, 228 aa, Nicotiana tabacum
  N. tabacum RieskeFeS protein
MASSTLSPVTQLCSSKSGLSSVSQCLLLKPMKINSHGLGKDKRMKVKCMATSIPADDRVPDMEKRNLMNLLLLGALSLPTAGMLVPYATFFAPPGSGGGSGGTPAKDALGNDVIASEWLKTHPPGNRTLTQGLKGDPTYLVVENDGTLATYGINAVCTHLGCVVPFNAAENKFICPCHGSQYNNQGRVVRGPAPLSLALAHADIDDGKVVFVPWVETDFRTGEDPWWA

SEQ ID NO: 2 - DNA, 666 bp, Nicotiana tabacum
  N. tabacum PetC cDNA
atggcttcttctactctttctccagtaactcagctatgctcgagcaagagtggtttgtcttcagtttcacaatgtttgctactgaagccaatgaagattaacagtcatggattgggaaaggataagaggatgaaagtcaagtgcatggctacaagcattccagcagatgatagagtgcctgatatggaaaagaggaatctcatgaatttgcttcttttgggtgctctttctctacccactgctgggatgttggtaccttatgctactttctttgcaccacctgggtcagggggtggtagtggtggaacccctgccaaggatgcattaggtaatgatgtcattgcatctgaatggctcaaaactcatccacccggcaaccgaactctcacgcaaggactaaagggagatcctacttaccttgttgtggagaatgatggaacacttgcaacctatggtattaatgctgtgtgtactcaccttggttgtgttgtgccatttaatgctgctgagaacaagtttatttgcccctgccatggatctcaatataacaaccaaggaagagttgttagaggacctgctcctttgtccttggcattggctcatgctgacattgatgatgggaaggtggtgtttgtcccatgggttgaaacagacttcagaactggt

SEQ ID NO: 3 - DNA, 833 bp, Nicotiana tabacum
  N. tabacum PetC gene
aaatggcttcttctactctttctccagtaactcagctatgctcaagcaagagtggcttgtcttcagtttcacaatgtttgctagtgaagccaatgaagattaacagtcatggattgggaaaagataagaggatgaaagtgaaatgcatggctacaagtattccagcagatgatagagtgcctgatatggaaaagaggaatctcatgaatttgcttcttttgggtgctctttctctacccactgctgggatgttggtatcttatggtactttctttgtaccacctgggtcagggggtggtagtggtggaacccctgccaaggatgcattaggtaatgatgtcattgcatctgaatggctcaaaactcatccacctggcaaccgaactctcacgcaaggactaaagggagaccctacttaccttgttgtggagaatgatggaacagttgcaacctatggtattaatgctgtgtgtactcaccttggttgtgttgtgccatttaatgctgctgagaacaagtttatttgcccctgccatggatctcaatacaacaaccaaggaagagttgttagaggacctgctcccttgtccttggcattggctcatgctgatattgatgatgggaaggtggtgtttgtcccatgggttgaaacagacttcagaactggtgaagatccatggtgggcttagatctccttatcactatattatcctcttgtatctttgttacataaagcttatctcctttttatgaagcaaaaagaaatattcattttgatgatgtaactattgaaggataacctttgcagtcccataatgacattttttgtttaa

SEQ ID NO: 4 - DNA, 29 bp, Artificial Sequence
  RT-PCR Primer 1
caccatggcttcttctactctttctccag

SEQ ID NO: 5 - DNA, 24 bp, Artificial Sequence
  RT-PCR Primer 2
ctaagcccaccatggatcttcacc